European Patent Application EP 4 137 512 A1, published February 22, 2023. Title: Anti-GM2AP ANTIBODY AND APPLICATIONS THEREOF. Applicant: Vitae Biomedical Co., Ltd. The sequence listing filed with the application follows.

SEQUENCE LISTING (119 sequences)

SEQ ID NO: 1 - protein, 14 aa, synthetic construct
  REGION 1..14: note = GM2AP and one of the amino acids from position 1 to 14 is glycosylated with (GlcNAc)2Fuc(Man)3
PIIVPGNVTLSVVG

SEQ ID NO: 2 - protein, 193 aa, synthetic construct
  REGION 1..193: note = GM2AP and one of the amino acids from position 57 to 70 is glycosylated with (GlcNAc)2Fuc(Man)3
MQSLMQAPLLIALGLLLAAPAQAHLKKPSQLSSFSWDNCDEGKDPAVIRSLTLEPDPIIVPGNVTLSVMGSTSVPLSSPLKVDLVLEKEVAGLWIKIPCTDYIGSCTFEHFCDVLDMLIPTGEPCPEPLRTYGLPCHCPFKEGTYSLPKSEFVVPDLELPSWLTTGNYRIESVLSSSGKRLGCIKIAASLKGI

SEQ ID NO: 3 - protein, 193 aa, synthetic construct [sequence omitted]

SEQ ID NO: 4 - protein, 202 aa, synthetic construct
  REGION 1..202: note = GM2AP and one of the amino acids from position 57 to 70 is glycosylated with (GlcNAc)2Fuc(Man)3
MQSLMQAPLLIALGLLLAAPAQAHLKKPSQLSSFSWDNCDEGKDPAVIRSLTLEPDPIIVPGNVTLSVMGSTSVPLSSPLKVDLVLEKEVAGLWIKIPCTDYIGSCTFEHFCDVLDMLIPTGEPCPEPLRTYGLPCHCPFKEGTYSLPKSEFVVPDLELPSWLTTGNYRIESVLSSSGKRLGCIKIAASLKGIRHHHHHHHH

SEQ ID NO: 5 - protein, 113 aa, synthetic construct
  REGION 1..113: note = 21-2B5-F7 light chain variable region
DIVMTQTASSVYVTPGESVSISCRSTKSLLHSNGDTYLYWFLQRPGQSPQLLIYRMSNLAPGVPDRFSGGGSGTAFTLRISRVEAEDVGVYYLYATSTISFHVRCWDQAGAET

SEQ ID NO: 6 - protein, 120 aa, synthetic construct
  REGION 1..120: note = 21-2B5-F7 heavy chain variable region
EIQLQQSGAELVRPGTSVKISCMASGYSFTGYNMNWVRQSHGRSLEWIGNINPYFGSPNYNQKFKGKATLTLDRSSNTAYMQLNRVTSEDSAVYYCASRQLGLGDTMDYWGQGTSVTVSS

SEQ ID NO: 7 - protein, 107 aa, synthetic construct
  REGION 1..107: note = 21-4E3-C8-A light chain variable region
DIVMTQSHKFMSTSVGDRVTITCKASQDVSTAVGWYQQKPGQSPKLLIYWASTRHTGVPDRFTGSRFGTDYTLTISSVQAEDLALYYCQQHYITPWTFGGGTKLEIK

SEQ ID NO: 8 - protein, 119 aa, synthetic construct
  REGION 1..119: note = 21-4E3-C8-A heavy chain variable region
QVQLQQPGADFVKPGASVKLSCKASGYTFTSYWINWVKQRPGQGLEWIGNIYPGSGSTNYNEKFKNKATLTIDTSSSTAYMQLSSLTSDDSAVYYCSRSTLYSYDDGSWGQGTTLTVSS

SEQ ID NO: 9 - protein, 107 aa, synthetic construct
  REGION 1..107: note = 21-4E3-C8-A heavy chain variable region
DIQMTQSPSSLSASLGERVSLTCRASQEISGDLSWLQQKPDGTIKRLIYAASTLASGVPKRFSGSRSGSDYSLTISGLESEDFADYYCLQYVSYPFTFGSGTKLEIK

SEQ ID NO: 10 - protein, 117 aa, synthetic construct
  REGION 1..117: note = 21-4E3-C8-B light chain variable region
QIQLQQSGPELGKPGASVKISCKASDYTFTDFYISWVKQRPGQGLEWIGWIYPLDDHTKYNEKFKGKATLTVDISSNTVYMQLSSLTSEDSAVYFCARIYGYAMDYWGQGTSVTVSS

SEQ ID NO: 11 - protein, 107 aa, synthetic construct
  REGION 1..107: note = 21-2H9-G2 light chain variable region
DIQMTQSPSSLSASLGERVSLTCRASQEISGDLSWLQQKPDGTIKRLIYAASTLASGVPKRFSGSRSGTDYSLTISGLESEDFADYYCLQYVSYPFTFGSGTKLEIK

SEQ ID NO: 12 - protein, 119 aa, synthetic construct; identical to SEQ ID NO: 8
  REGION 1..119: note = 21-2H9-G2 heavy chain variable region

SEQ ID NO: 13 - protein, 107 aa, synthetic construct
  REGION 1..107: note = 21-4G4-B11 light chain variable region
EIVMTQSHNHVHISGRQGHHHLQGQSGCEYCCRLVSTETRAISITTDFTGHPPGTLESLIAFTGSRSGTDYTLTISSVQAEDLALYYCQQHYITPWTFGGGTKLEIK

SEQ ID NO: 14 - protein, 117 aa, synthetic construct; identical to SEQ ID NO: 10
  REGION 1..117: note = 21-4G4-B11 heavy chain variable region

SEQ ID NO: 15 - protein, 113 aa, synthetic construct
  REGION 1..113: note = 21-4B10-E1 light chain variable region
DIVMTSETHLCICHSWRVSLHLLQVYIESPAIIWRHLFVLVPTEARPVSSAPDISDVQPCPRSPTQVQWRWVRNCFHTENQISGGTGCGCLLLYATSTISFHVRCWDQAGAET

SEQ ID NO: 16 - protein, 120 aa, synthetic construct; identical to SEQ ID NO: 6
  REGION 1..120: note = 21-4B10-E1 heavy chain variable region

SEQ ID NO: 17 - protein, 107 aa, synthetic construct
  REGION 1..107: note = 22-2E9-G12 light chain variable region
DIVMTQSQKFMSTSIGDRVSVTCKASQNVNTNIAWYQQKPGQSPKALIYSASYRYSGVPDRFTGSGSGTDFTLTISSVQSEDLAEYFCQQYIGYPYTFGGGTKLEIK

SEQ ID NO: 18 - protein, 120 aa, synthetic construct
  REGION 1..120: note = 22-2E9-G12-A heavy chain variable region
QVQLQQPGATLVRPGASVKLSCKASGYTFINYWINWVKWRPGQGLEWIGNINPNCGVTKYNEQIKSEATLTVDKSSSIAYMQLSSLTSEDSAVYYCPHLLLRWLLHVPFAMVYWGQGTSV

SEQ ID NO: 19 - protein, 118 aa, synthetic construct
  REGION 1..118: note = 22-2E9-G12-B heavy chain variable region
EVQLVETGGGLVQPQGSLKLSCAASGFNFNTYAMNWVRQAPGKGLEWVARIRTKSNSYATYYADSVKDRFIISRDDSQSMLYLQMNNLKTEDTAIFYCVVTYWGFIYWGQGTLVTVSA

SEQ ID NO: 20 - protein, 112 aa, synthetic construct
  REGION 1..112: note = 22-3E6-B11 light chain variable region
DVVMTQTPLTLSVTIGQPASISCKSSQSLLYSDRKTYLNWLFQRPGQSPKRLIYLVSKLDSGVPDRFTGSGSGTDFTLKISRVEAEDLGIYYCWQGTHFPQTFGGGTKLEIK

SEQ ID NO: 21 - protein, 115 aa, synthetic construct
  REGION 1..115: note = 22-3E6-B11 heavy chain variable region
EVQLQQSGPELVKPGASVKMSCKASGYSFTAYYIHWMKQSPEKSLEWIGEINPSTDDTTYNQNFKSKATLTVDRSSRTAYMQLRSLTSEDSAVYFCARYGEGAYWGQGTLVTVSA

SEQ ID NO: 22 - protein, 112 aa, synthetic construct
  REGION 1..112: note = 22-4B11-B9 light chain variable region
DVVMTQIPLTLSVIIGQPASISCKSSQSLLYSDGKTYLNWLLQRPGQSPKRLIYLVSKLDSGVSDRFTGSGSGTDFTLKISRVEAEDLGVYYCWQGTHFPQTYGGGTKLEIK

SEQ ID NO: 23 - protein, 115 aa, synthetic construct
  REGION 1..115: note = 22-4B11-B9 heavy chain variable region
EVQLQQSGPELVKPGASVKISCKASGYSFTGFPHALGEAKSTKEPTVDWRDISIYWWYYLQSEVQGQGHIDCRQILQYSLYATQEPDITRLCSLLLCKIRRGGLLGPRDSGLCLC

SEQ ID NO: 24 - protein, 106 aa, synthetic construct
  REGION 1..106: note = 22-5B1-B2 light chain variable region
IVMTQSPKSMSMSVGERVTLSCKASENVGTYVSWYQQKPEQSPKLLIYGASNRYTGVPDRFTGSGSATDFTLTISSVQAEDLADYHCGQSYSYPLTFGAGTKLELK

SEQ ID NO: 25 - protein, 115 aa, synthetic construct
  REGION 1..115: note = 22-5B1-B2 heavy chain variable region
EVQMQQSGPELVKPGASVEISCKASGYSFTGYYIHWVKQSPEKNLEWIGEVNPISGGTTYNQRFKAKATLNVDTLSNTAYMQLKSLTSEDSAVYFCARYGATDYWGQGTSVTVSS

SEQ ID NO: 26 - protein, 115 aa, synthetic construct
  REGION 1..115: note = 22-5F2-E10 light chain variable region
EVQLQQSGPELVKPGASVKISCKASGYSFTGYYIHWVRRSPEKSLAWIGEINPTTGGTSYNQKFRAKATLTVDTSSSTAYIQLKSLTSEDSAIYYCARYGEGAYWGQGTLVTVSA

SEQ ID NO: 27 - protein, 113 aa, synthetic construct
  REGION 1..113: note = 22-5F2-E10 heavy chain variable region
DVVLTQTPLTLSVTFGQPASISCKSSQSLFIITWKDIFVFGCYRGQASLQSAISFWCLNWTLESLTGSVAVDQGQISHTRSTEWRLRIWEFIIAGKVHIFLRRTVEAPCWKSN

SEQ ID NO: 28 - DNA, 737 bp, synthetic construct
  misc_feature 1..737: note = 21-2B5-F7 light chain variable region
  source 1..737: mol_type = other DNA
gttagatctgtgagcgagctgcgtagaatgagttcctggcgctgcttgtgctctggatccctggagccattggggatattgtgatgactcagactgcatcctctgtatatgtcactcctggagagtcagtctccatctcctgcaggtctactaagagtctcctgcatagtaatggcgacacttatttgtattggttcctacagaggccaggccagtctcctcagctcctgatatatcggatgtccaaccttgccccaggagtccctgacaggttcagtggcggtgggtcaggaactgctttcacactgagaatcagtagagtggaggctgaggatgtgggtgtttattacctgtatgcaacatcttgaatatcctttcacgttcggtgctgggaccaagctggagctgaaacgggctgatgttgcaccaactgtatccatcttcccaccatccagtgagcagttaacatctggaggtgcctcagtcgtgtgcttcttgaacaacttctaccccaaagacatcaatgtcaagtggaagattgatggcagtgaacgacaaaatggcgtcctgaacagttggactgatcaggacagcaaagacagcacctacagcatgagcagcaccctcacgttgaccaaggacgagtatgaacgacataacagctatacctgtgaggccactcacaagacatcaacttcaccccattgtcaagagcttcaacaggatgagtgtacgcg

SEQ ID NO: 29 - DNA, 730 bp, synthetic construct
  misc_feature 1..730: note = 21-2B5-F7 heavy chain variable region
  source 1..730: mol_type = other DNA
tacaaagtaaccactcaaaggataaaataatcgcgaatttgccccccccaagagacaacgacgaagattggggtcatcctcttccttctgtcagtaactgcaggtgtccactctgagatccagctgcaacagtctggagctgagctggtgaggcctgggacttcagtgaagatatcctgcatggcttctggttactcattcactggctacaatatgaactgggtgaggcaaagccatggaaggagccttgagtggatcggaaatattaatccttactttggtagtcctaactacaatcagaagttcaagggcaaggccacattgactttagacagatcctccaacacagcctacatgcagctcaacagagtgacatctgaggactctgcagtctactactgtgcatcaaggcagctcgggctgggagatactatggactactggggtcaaggaacctcagtcaccgtctcctcagccaaaacaacagccccatcggtctatccactggcccctgtgtgtggagatacaagtggctcctcggtgactctaggatgcctggtcaagggttatttccctgagccagtgaccttgacctggaactctggatccctgtccagtggtgtgcacaccttcccagctgtcctgcagtctgacctctacaccctcagcagctcagtgactgtaacctcgagcacctggcccagccagtccatcacctgcaattgtcgct

SEQ ID NO: 30 - DNA, 651 bp, synthetic construct
  misc_feature 1..651: note = 21-4E3-C8-A light chain variable region
  source 1..651: mol_type = other DNA
gtgtttctccggttgtctggtgttgacggagacattgtgatgacccagtctcacaaattcatgtccacatcagtgggagacagggtcaccatcacctgcaaggccagtcaggatgtgagtactgctgtaggctggtatcaacagaaaccagggcaatctcctaaactactgatttactgggcatccacccggcacactggagtccctgatcgcttcacaggcagtagatttgggacagactatactctcaccatcagcagtgtgcaggctgaagacctggcactttattactgtcagcaacattatatcactccgtggacgttcggtggaggcaccaagctggaaatcaaacgggctgatgctgcaccaactgtatccatcttcccaccatccagtgagcagttaacatctggaggtgcctcagtcgtgtgcttcttgaacaacttctaccccaaagacatcaatgtcaagtggaagattgatggcagtgaacgacaaaatggcgtcctgaacagttggactgatcaggacagcaaagacagcacctacagcatgagcagcaccctcacgttgaccaaggacgagtatgaacgacataacagctatacctgtgaggccactcacaagaccacaacttcacccattcaacgg

SEQ ID NO: 31 - DNA, 658 bp, synthetic construct
  misc_feature 1..658: note = 21-4E3-C8-A heavy chain variable region
  source 1..658: mol_type = other DNA
cgacagtctttttggttgcagcagctacaggtgtccactcccaggtccaactgcagcagcctggtgctgactttgtgaagcctggggcctcagtgaagctgtcctgcaaggcttctggctacactttcaccagctactggataaactgggtgaagcagaggcctggacaaggccttgagtggattggaaatatttatcctggtagcggtagtactaactacaatgagaagttcaagaacaaggccacactgactatagacacatcctccagcacagcctacatgcagctcagcagcctgacatctgacgactctgcggtctactactgttcaagatcaaccctctatagttacgacgacggctcttggggccaaggcaccactctcacagtctcctcagccaaaacgacacccccatctgtctatccactggcccctggatctgctgcccaaactaactccatggtgaccctgggatgcctggtcaagggctatttccctgagccagtgacagtgacctggaactctggatccctgtccagcggtgtgcacaccttcccagctgtcctgcagtctgacctctacactctgagcagctcagtgactgtcccctccagcacctggcccagcgagaccgtcacctgcaacgtgcccctccc

SEQ ID NO: 32 - DNA, 653 bp, synthetic construct
  misc_feature 1..653: note = 21-4E3-C8-B light chain variable region
  source 1..653: mol_type = other DNA
tgttgctctggtttccaggtatcagatgtgacatccagatgacgcagtctccatcctccttatctgcctctctgggagaaagagtcagtctcacttgtcgggcaagtcaggaaattagtggtgacttaagctggcttcagcagaaaccagatggaactattaaacgcctgatatacgccgcatccactttagcttctggtgtcccaaaaaggttcagtggcagtaggtctgggtcagattattctctcaccatcagcggccttgagtctgaagattttgcagactattactgtctacaatatgttagttatccattcacgttcggctcggggacaaagttggaaataaaacgggctgatgctgcaccaactgtatccatcttcccaccatccagtgagcagttaacatctggaggtgcctcagtcgtgtgcttcttgaacaacttctaccccaaagacatcaatgtcaagtggaagattgatggcagtgaacgacaaaatggcgtcctgaacagttggactgatcaggacagcaaagacagcacctacagcatgagcagcaccctcacgttgaccaaggacgagtatgaacgacataacagctatacctgtgaggccacttcacatagacagcaaatctcacccattcaacag

SEQ ID NO: 33 - DNA, 653 bp, synthetic construct
  misc_feature 1..653: note = 21-4E3-C8-B heavy chain variable region
  source 1..653: mol_type = other DNA
ttgaacttgccattcctcctgtcaggaactgcaggtgtccattgccagatccagctgcagcagtctggacctgaactggggaagcctggggcttcagtgaagatatcctgcaaggcttctgactacaccttcactgacttctatataagttgggtgaaacagaggcctggacagggacttgagtggattggatggatttatcctttagacgatcatactaagtacaatgagaagttcaagggcaaggccacattgactgtagacatatcctccaacacagtctacatgcagctcagcagcctgacctctgaggactctgcggtctatttctgtgccagaatctatggatatgctatggactactggggtcaaggaacctcagtcaccgtctcctcagccaaaacaacagccccatcggtctatccactagcccctgtgtgtggagatacaactggctcctcggtgactttaggatgcctggtcaagggttatttccctgagccagtgaccttgacctggaactctggattcctgtccagtggtgtgcacacctttccagctgtcctgcagtctgacctctacaccctcagcagctcagcgactgtaacctcgagcacctggcccagccataccatacctgcagacggtccccc

SEQ ID NO: 34 - DNA, 751 bp, synthetic construct
  misc_feature 1..751: note = 21-2H9-G2 light chain variable region
  source 1..751: mol_type = other DNA
gcggtcatctgcacgatcatgagggtacctcgctcacgtgctttaagattcttgtcagctctggtttccaggtatcagatgtgacatccagatgacccagtctccatcctccttatctgcctctctgggagaaagagtcagtctcacttgtcgggcaagtcaggaaattagtggtgacttaagctggcttcagcagaaaccagatggaactattaaacgcctgatctacgccgcatccactttagcttctggtgtcccaaaaaggttcagtggcagtaggtctgggtgagattattctctcaccatcagcggccttgagtctgaagattttgcagactattactgtctacaatatgttagttatccattcacgttcggctcggggacaaagttggaaataaaacgggctgatgctgcaccaactgtatccatcttcccaccatccagtgagcagttaacatctggaggtgcctcagtcgtgtgcttcttgaacaacttctaccccaaagacatcaatgtcaagtggaagattgatggcagtgaacgacaaaatggcgtcctgaacagttggactgatcaggacagcaaagacagcacctacagcatgagcagcaccctcacgttgaccaaggacgagtatgaacgacataacagctatacctgtgaggccactcacaagacatcagttttcccccattatcagagggctttcaccaggaatgagtgtagcccgccaaaaaaaaaaaaaaac

SEQ ID NO: 35 - DNA, 660 bp, synthetic construct
  misc_feature 1..660: note = 21-2H9-G2 heavy chain variable region
  source 1..660: mol_type = other DNA
cgtctgtctttttggttgcagcagctacaggtgtccactcccaggtccaactgcagcagcctggtgctgactttgtgaagcctggggcctcagtgaagctgtcctgcaaggcttctggctacactttcaccagctactggataaactgggtgaagcagaggcctggacaaggccttgagtggattggaaatatttatcctggtagcggtagtactaactacaatgagaagttcaagaacaaggccacactgactatagacacatcctccagcacagcctacatgcagctcagcagcctgacatctgacgactctgcggtctactactgttcaagatcaaccctctatagttacgacgacggctcttggggccaaggcaccactctcacagtctcctcagccaaaacgacacccccatctgtctatccactggcccctggatctgctgccccaaaactaactccatggtgaccctgggatgcctggtcaagggctatttccctgagccagtgacagtgacctggaactctggatccctgtccagcggtgtgcacaccttcccagctgtcctgcagtctgacctctacactctgagcagctcagtgactgtcccctccagcacctggcccagcgagaccgtcacctgcaacgtgcccgtcca

SEQ ID NO: 36 - DNA, 795 bp, synthetic construct
  misc_feature 1..795: note = 21-4G4-B11 light chain variable region
  source 1..795: mol_type = other DNA
gactagagcacgtggtgtctggtgttgacggagaaattgtgatgacccagtctcacaatcatgtccacatcagtgggagacagggtcaccatcacctgcaaggccagtcaggatgtgagtactgctgtaggctggtatcaacagaaaccagggcaatctcctaaactactgattttactgggcatccacccggcacactggagtccctgatcgctttcacaggcagtagatctgggacagactatactctcaccatcagcagtgtgcaggctgaagacctggcactttattactgtcagcaacattatatcactccgtggacgttcggtggaggcaccaagctggaaatcaaacgggctgatgctgcaccaactgtatccatcttcccaccatccagtgagcagttaacatctggaggtgcctcagtcgtgtgcttcttgaacaccttctaccccaaagacatcaatgtcaagtggaagattgatggcagtgaacgacaaaatggcgtcctgaacagttggactgatcaggacagcaaagacagcacctacagcatgagcagcaccctcacgttgaccaaggacgagtatgaacgacataacagctatacctgtgaggccactcacaagacatcaacttcacccattgtcaagagcttcaacaggaatgagtgtagggggggggaaaaaaaaaaaaaaaaaaaaaaggcggaggggacgcggataaaaataaccgttagcatgacttaagtgcgtaacatattcaatctttctttccgcgggggcgggaaagagg

SEQ ID NO: 37 - DNA, 666 bp, synthetic construct
  misc_feature 1..666: note = 21-4G4-B11 heavy chain variable region
  source 1..666: mol_type = other DNA
catgaatggagctgggtcattctcttcctcctgtcaggaactgcaggtgtccattgccagatccagctgcagcagtctggacctgaactggggaagcctggggcttcagtgaagatatcctgcaaggcttctgactacaccttcactgacttctatataagttgggtgaaacagaggcctggacagggacttgagtggattggatggatttatcctttagacgatcatactaagtacaatgagaagttcaagggcaaggccacattgactgtagacatatcctccaacacagtctacatgcagctcagcagcctgacctctgaggactctgcggtctatttctgtgccagaatctatggatatgctatggactactggggtcaaggaacctcagtcaccgtctcctcagccaaaacaacagccccatcggtctatccactggcccctgtgtgtggagatacaactggctcctcggtgactctaggatgcctggtcaagggttatttccctgagccagtgaccttgacctggaactctggatccctgtccagtggtgtgcacaccttcccagctgtcctgcagtctgacctctacaccctcagcagctcagtgactgtaacctcgagcacctggcccagccagtccatcacctgcaatggcccgcag

SEQ ID NO: 38 - DNA, 720 bp, synthetic construct
  misc_feature 1..720: note = 21-4B10-E1 light chain variable region
  source 1..720: mol_type = other DNA
gccccccttttttatgggggggggaacttgcctcagctcagttccttgggctgcttgtgctctggatccctggagccattggggatattgtgatgacttcagaaactcacctctgtatatgtcactcctggagagtcagtctccatctcctgcaggtctactaagagtctcctgcatagtaatggcgacacttatttgtattggttcctacagaggccaggccagtctcctcagctcctgatatatcggatgtccaaccttgccccaggagtccctgacaggttcagtggcggtgggtcaggaactgctttcacactgagaatcagtagagtggaggctgaggatgtgggtgtttattactgtatgcaacatcttgaatatcctttcacgttcggtgctgggaccaagctggagctgaaacgggctgatgttgcaccaactgtatccatcttcccaccatccagtgagcagttaacatctggaggtgcctcagtcgtgtgcttcttgaacaacttctaccccaaagacatcaatgtcaagtggaagattgatggcagtgaacgacaaaatggcgtcctgaacagttggactgatcaggacagcaaagacagcacctacagcatgagcagcaccctcacgttgaccaaggacgagtatgaacgacataacagctaacctgtgaggccactcacaagacatcaacttcacccattcaacggg

SEQ ID NO: 39 - DNA, 687 bp, synthetic construct
  misc_feature 1..687: note = 21-4B10-E1 heavy chain variable region
  source 1..687: mol_type = other DNA
agccttccccccccaaagggaggggtgaccttgctattccttctgtcagtaactgcaggtgtccactctgagatccagctgcaacagtctggagctgagctggtgaggcctgggacttcagtgaagatatcctgcatggcttctggttactcattcactggctacaatatgaactgggtgaggcaaagccatggaaggagccttgagtggatcggaaatattaatccttactttggtagtcctaactacaatcagaagttcaagggcaaggccacattgactttagacagatcctccaacacagcctacatgcagctcaacagagtgacatctgaggactctgcagtctactactgtgcatcaaggcagctcgggctgggagatactatggactactggggtcaaggaacctcagtcaccgtctcctcagccaaaacaacagccccatcggtctatccactagcccctgtgtgtggagatacaagtggctcctcggtgactttaggatgcctggtcaagggttatttccctgagccagtgaccttgacctggaactctggatccctgtccagtggtgtgcacaccttcccagctgtcctgcagtctgacctctacaccctcagcagctcagtgactgtaacctcgagcacctggcccagctcagtccgtcgcactgcttgctgttca

SEQ ID NO: 40 - DNA, 680 bp, synthetic construct
  misc_feature 1..680: note = 22-2E9-G12 light chain variable region
  source 1..680: mol_type = other DNA
ggtcatactgctgtggtgtctggtgttgatggagacattgtgatgacccagtctcaaaaattcatgtccacatcaataggagacagggtcagcgtcacctgcaaggccagtcagaatgtgaatactaatatagcctggtatcaacagaaaccaggacagtctcctaaagcactgatttactcggcttcctaccgctatagtggagtccctgatcgcttcacaggcagtggatctgggacagatttcactctcaccatcagcagtgtgcagtctgaggacttggcagaatatttctgtcagcaatatatcggctatccgtacacgttcggaggggggaccaagctggaaataaaacgggctgatgctgcaccaactgtatccatcttcccaccatccagtgagcagttaacatctggaggtgcctcagtcgtgtgcttcttgaacaacttctaccccaaagacatcaatgtcaagtggaagattgatggcagtgaacgacaaaatggcgtcctgaacagttggactgatcaggacagcaaagacagcacctacagcatgagcagcaccctcacgttgaccaaggacgagtatgaacgacataacagctatacctgtgaggccactcacaagacatcaacttcacccattgtcaagagcttcaacaggaatgagtgtaaccc

SEQ ID NO: 41 - DNA, 676 bp, synthetic construct
  misc_feature 1..676: note = 22-2E9-G12-A heavy chain variable region
  source 1..676: mol_type = other DNA
gggtcatctcttcttggtagcaactgctacaggtgtccactcccaggtccaactgcagcagcctggggcttgactggtgaggcctggggcttcagtgaagttgtcctgcaaggcttctggctacaccttcatcaactactggataaactgggtgaagtggaggcctggacaaggccttgagtggattggaaatattaatcctaattgtggtgttactaagtacaatgagcagatcaagagcgaggccacactgactgtagacaaatcctccagcatagcctacatgcaactcagcagcctgacatctgaggactctgcggtctattactgtcctcatttattactacgatggttgctacacgtcccctttgctatggtctactggggtcaaggaacctcagtcaccgtctcctcagccaaaacaacagccccatcggtctatccactggcccctgtgtgtggagatacaagtggctcctcggtgactctaggatgcctggtcaagggttatttccctgagccagtgaccttgacctggaactctggatccctgtccagtggtgtgcacaccttcccagctgtcctgcagtctgacctctacaccctcagcagctcagtgactgtaacctcgagcacctggcccagccagtccatcacctgcaattggccctcccca

SEQ ID NO: 42 - DNA, 726 bp, synthetic construct
  misc_feature 1..726: note = 22-2E9-G12-B heavy chain variable region
  source 1..726: mol_type = other DNA
gtggggtcaatatacattgtcatgctgttagggctgaagtgggttttctttgttgttttttatcaaggtgtgcattgtgaggtgcagcttgttgagactggtggaggattggtgcagcctcaagggtcattgaaactctcatgtgcggcctctggattcaacttcaatacctatgccatgaactgggtccgccaggctccaggaaagggtttggaatgggttgctcgcataagaactaaaagtaattcttatgcaacatattatgccgattcagtgaaagacaggttcatcatctccagagatgattcccaaagcatgctctatctgcaaatgaacaacttgaaaactgaggacacagccatattttactgtgtggttacctactgggggtttatttactggggccaagggactctggtcactgtctctgcagccaaaacaacagccccatcggtctatccactggcccctgtgtgtggagatacaagtggctcctcggtgactctaggatgcctggtcaagggttatttccctgagccagtgaccttgacctggaactctggatccctgtccagtggtgtgcacaccttcccagctgtcctgcagtctgacctctacaccctcagcagctcagtgactgtaacctcgagcacctggcccagccagtccatcacctgcaatgtggcccaacacggcaagcagcacccgtaaaaaaaaaaatttggt

SEQ ID NO: 43 - DNA, 788 bp, synthetic construct
  misc_feature 1..788: note = 22-3E6-B11 light chain variable region
  source 1..788: mol_type = other DNA
agctcaacaacaaaaaaaacaaaaaacaaaaaaagataaaatctacacgtgacgggagttggggggagaggcagtgctcttttttttaggggggggggacactagttgcctgttaggctgttggtgctctggattcgggaaaccaacggtgatgttgtgatgacccagactccactcactttgtcggttaccattggacaaccagcctccatatcttgcaagtcaagtcagagcctcttatatagtgatagaaagacatatttgaattggttgtttcagaggccaggccagtctccaaagcgcctaatctatctggtctctaaactggactctggagtccctgacaggttcactggcagtggatcagggacagatttcacactgaaaatcagcagagtggaggctgaggatttgggaatttattattgctggcaaggtacacattttcctcagacgttcggtggaggcaccaagttggaaatcaaacgggctgatgctgcaccaactgtatccatcttcccaccatccagtgagcagttaacatctggaggtgcctcagtcgtgtgcttcttgaacaacttctaccccaaagacatcaaagtcaaagtggaagattgatggcagtgaacgacaaaatggcgtcctgaacagttggactgatcaggacagcaaagacagcacctacagcatgagcagcaccctcacgttgaccaaggacgagtatgaacgacataacagctatacctgtgaggccactcacaaagagatcaaatttcacccattcaacg

SEQ ID NO: 44 - DNA, 657 bp, synthetic construct
  misc_feature 1..657: note = 22-3E6-B11 heavy chain variable region
  source 1..657: mol_type = other DNA
gtaggaagctgggtttcctcttaatcctgtcagtaactacaggtgtcccactctgaggtccagctgcagcagtctggacctgagctggtgaagcctggggcttcagtgaagatgtcctgcaaggcttctggttactcattcactgcctattacatacactggatgaagcaaagtcctgaaaagagccttgagtggattggagagattaatcctagcactgatgacacaacctacaaccagaacttcaagtccaaggccacattgactgtagacaggtcctccagaacagcctacatgcaactcaggagcctgacatctgaggactctgcagtctatttctgtgcaagatacggcgagggggcttactggggccaagggactctggtcactgtctctgcagccaaaacaacagccccatcggtctatccactggcccctgtgtgtggagatacaagtggctcctcggtgactctaggatgcctggtcaagggttatttccctgagccagtgaccttgacctggaactctggatccctgtccagtggtgtgcacaccttcccagctgtcctgcagtctgacctctacaccctcagcagctcagtgactgtaacctcgagcacctggcccagccagaccatcacctgcaatgtgctcgct

SEQ ID NO: 45 - DNA, 889 bp, synthetic construct
  misc_feature 1..889: note = 22-4B11-B9 light chain variable region
  source 1..889: mol_type = other DNA
gcatcgccttaacacgctcgtccttatttgctacactgaaggtgcccgtacgctttcgggtatcgttgacatgaaatgcccagtcatgccgttggggtaagcgttgaccactgaagcttgacagttaagcctttgggtaatcgttgaacaataaaagatgccagtttagcctttggggcttttatttatagggcgggaaaacactagtgcctgttaggctgttggtgctctggattcgggaaaccaacggtgatgttgtgatgacccagattccactcactttgtcggttatcattggacaaccagcctccatctcttgcaagtcaagtcagagcctcttatatagtgatggaaagacatatttgaattggttgttacagaggccaggccagtctccaaagcgcctaatctatctggtgtctaaactggactctggagtctctgacaggttcactggcagtggatcagggacagatttcacactgaaaatcagcagagtggaggctgaggatttgggagtttattattgctggcaaggtacacattttccgcagacgtacggtggaggcaccaagctggaaatcaaacgggctgatgctgcaccaactgtatccatcttcccaccatccagtgagcagttaacatctggaggtgcctcagtcgtgtgcttcttgaacaacttctaccccaaagacatcaatgtcaagtggaagattgatggcagtgaacgacaaaatggcgtcctgaacagttggactgatcaggacagcaaagacagcacctacagcatgagcagcaccctcacgttgaccaaggacgagtatgaacgacataacagctatacctggaggcccgcgtcgacacatcagcgccacctcagtgccaaggg

SEQ ID NO: 46 - DNA, 757 bp, synthetic construct
  misc_feature 1..757: note = 22-4B11-B9 heavy chain variable region
  source 1..757: mol_type = other DNA
acggtaatgaaagaagggggtggacctgggttttttttttgccgttttttttccaccttttttaaaatttggggttaaaaccccccccctttttcaatgtagaacctgggctttattttaatcctgtcagtaactacaggtgtccactctgaggtccagctgcaacagtctggacctgagctggtgaagcctggggcgtcagtgaagatttcctgcaaggcttctggttactcattcactggttttcctcatgcactgggtgaagcaaagtcctgaaaagagccttgagtggattggagagattaatcctagtactggtggtactacctacaatcagaggttcaaggccaaggccacattgactgtagacaaatcctacagtacagcctatatgcaactcaggagcctgacatctgaagactctgcagtctattactgtgcaagatacggcgagggggcttactggggccaagggactctggtctctgtctctgcggccaaaacaacagccccatcggtctatccactggcccctgtgtgtggagatacaagtggctcctcggtgactctaggatgcctggtcaagggttatttccctgagccagtgaccttgacctggaactctggatccctgtccagtggtgtgcacaccttcccagctgtcctgcagtctgacctctacaccctcagcagctcagtgactgtaacctcgagcacctggcccagccagtccatcacctgcatataatcttgcaag

SEQ ID NO: 47 - DNA, 1013 bp, synthetic construct
  misc_feature 1..1013: note = 22-5B1-B2 light chain variable region
  source 1..1013: mol_type = other DNA
ctgttcatgcctgcagacatgacagtcagaagatgagttacatcatcgagaatgaatagcttatgatattcgattgttcgataacaatgcatgacaaacaagctagtatgattgatcctacggtcactcagatggttactatgcaagacgaaagaagacagatgctacatatcaaactctcttggtgcaggtcatttacttccttttttgatgagtactttgcataaagttcctagagggcagaccagctgttccatgatttataaacctaggcccttctccacggagatctcaaaagcatcataacttcactgggggggcccccctcaaatgtgggggggggggaggacgccttatatccttgctgttctggttatatggtgctgatgggaacattgtaatgacccaatctcccaaatccatgtccatgtcagtaggagagagggtcaccttgagctgcaaggccagtgagaatgtgggtacttatgtatcctggtatcaacagaaaccagagcagtctcctaaactgctgatatacggggcatccaaccggtacactggggtccccgatcgcttcacaggcagtggatcagcaacagatttcactctgaccatcagcagtgtgcaggctgaagaccttgcagattatcactgtggacagagttacagctatccgctcacgttcggtgctgggaccaagctggagctgaaacgggctgatgctgcaccaactgtatccatcttcccaccatccagtgagcagttaacatctggaggtgcctcagtcgtgtgcttcttgaacaacttctaccccaaagaccatcaaagtcaaagtggaagattgatggcagtgaacgacaaaatggcgtcctgaacagttggactgatcaggacagcaaagacagcacctacagcatgagcagcaccctcacgttgaccaaggacgagtatgaacgacataacagctatacctgtgaggccactcacaagacatcaacttcacccattcaagg

SEQ ID NO: 48 - DNA, 1066 bp, synthetic construct
  misc_feature 1..1066: note = 22-5B1-B2 heavy chain variable region
  source 1..1066: mol_type = other DNA
gtattatgtgaggtgtcttttcctggtggcatcttcatcctattgtcttctgtcaacgtgattttcttttatacagcttctgtactcagtatttatatattagtatgcatttatttctttcttatctgttttcgtaattacgtggggttaatcggactgttagaaagctgtgttgagatttgctttttatgtttgctttaattaggatgctattgatctgagtttgatatgtaattatacagcatccatttcgaatggtaacagtaagctcttatggatttcgacaggattcatgtacaaaggttttagcaatggtgcttcctgggttctatgctggagtctcttgttgtaattggtggaagatttttaaacattcgctaaaaagcagcaaagaataataagaaaaaggtgttgaactgggtctttgttttaatcctgtcagtaactacaggtgtccactctgaggtccagatgcagcagtctggacctgagctggtgaagcctggggcttcagtggagatttcctgcaaggcttctggttactcattcactggctattacatacactgggtgaagcaaagtcctgaaaagaaccttgaatggattggagaggttaatcctattagtggtggtactacctacaaccagagattcaaggccaaggccacattgaatgtggacacattatccaacacagcctacatgcagctcaagagcctgacatctgaggactctgcagtctatttctgtgcacgatacggggctacggactattggggtcaaggaacctcagtcaccgtctcctcagccaaaacaacagccccatcggtctatccactggcccctgtgtgtggagatacaagtggctcctcggtgactctaggatgcctggtcaagggttatttccctgagccagtgaccttgacctggaactctggatccctgtccagtggtgtgcacaccttcccagctgtcctgcagtctgacctctacaccctcagcagctcagtgactgtaacctcgagcacctggcccagccagtccatctaccgctatagaacgtgca

SEQ ID NO: 49 - DNA, 767 bp, synthetic construct
  misc_feature 1..767: note = 22-5F2-E10 heavy chain variable region
  source 1..767: mol_type = other DNA
ttacaaaataaacagataagcgtttccattaaacataaaaaatttatggtaacgctttttttttttggggggggggaaccaagttgcctgttaggctgttggtgctctggattcgggataccaacggtgatgttgtgctgacccagactccactcactttgtcggttacctttggacaaccagcctccatctcttgcaagtcaagtcagagcctctttatatagtgatggaaagacatatttgtatttggttgttacagaggccaggccagtctccaaagcgcctaatctttctggtgtctaaactggactctggagtccctgacaggttcagtggcagtggatcagggacagatttcacactgaagatcaacagagtggaggctgaggatttgggaatttattattgctggcaaggtacacattttcctcagacgtacggtggaggcaccatgctggaaatcaaacgggctgatgctgcaccaactgtatccatcttcccaccatccagtgagcagttaacatctggaggtgcctcagtcgtgtgcttcttgaacaacttctaccccaaagacatcaatgtcaagtggaagattgatggcagtgaacgacaaaatggcgtcctgaacagttggactgatcaggacagcaaagacagcacctacagcatgagcagcaccctcacgttgaccaaggacgagtatgaacgacataacagctatacctgtgaggtcactcacaagactatcaacttcacccattcaagtg

SEQ ID NO: 50 - DNA, 737 bp, synthetic construct
  misc_feature 1..737: note = 22-5F2-E10 light chain variable region
  source 1..737: mol_type = other DNA
acatacaatcaatcgaacatacacaaaacattacccctcttataaaacatttcgttacacctccctactcccccccgatgagtcgccgggctttattttaaatcctgtcagtaactacaggtgtccactctgaggtccagctgcagcagtctggacctgaactggtgaagcctggggcttcagtgaagatatcttgcaaggcttctggttactcattcactggctactacatacactgggtgaggcgaagtcctgaaaagagccttgcgtggattggagagattaatcctaccactggtggtacttcctacaaccagaaattcagggccaaggccacattgactgtagacacgtcgtccagcacagcctatattcagctcaagagcctgacatctgaggactctgcaatctattactgtgcaagatacggcgagggggcttactggggccaagggactctggtcactgtctctgcagccaaaacaacagccccatcggtctatccactggcccctgtgtgtggagatacaagtgggctccctcggtgactctaggatgcctggtcaagggttatttccctgagccagtgaccttgacctggaactctggatccctgtccagtggtgtgcacaccttcccagctgtcctgcagtctgacctctacaccctcagcagctcagtgactgtaacctcgagcacctggcccagccagtccatcacctcatacgacctgctaa

SEQ ID NO: 51 - protein, 11 aa, synthetic construct
  REGION 1..11: note = 21-2B5-F7 LCDR1
KSLLHSNGDTY

SEQ ID NO: 52 - skipped

SEQ ID NO: 53 - protein, 9 aa, synthetic construct
  REGION 1..9: note = 21-2B5-F7 LCDR3
YATSTISFH

SEQ ID NO: 54 - protein, 8 aa, synthetic construct
  REGION 1..8: note = 21-2B5-F7 HCDR1
GYSFTGYN

SEQ ID NO: 55 - protein, 8 aa, synthetic construct
  REGION 1..8: note = 21-2B5-F7 HCDR2
INPYFGSP

SEQ ID NO: 56 - protein, 13 aa, synthetic construct
  REGION 1..13: note = 21-2B5-F7 HCDR3
ASRQLGLGDTMDY

SEQ ID NO: 57 - protein, 6 aa, synthetic construct
  REGION 1..6: note = 21-4E3-C8-A LCDR1
QDVSTA

SEQ ID NO: 58 - skipped

SEQ ID NO: 59 - protein, 10 aa, synthetic construct
  REGION 1..10: note = 21-4E3-C8-A LCDR3
QQHYITPWTF

SEQ ID NO: 60 - protein, 8 aa, synthetic construct
  REGION 1..8: note = 21-4E3-C8-A HCDR1
GYTFTSYW

SEQ ID NO: 61 - protein, 8 aa, synthetic construct
  REGION 1..8: note = 21-4E3-C8-A HCDR2
IYPGSGST

SEQ ID NO: 62 - protein, 12 aa, synthetic construct
  REGION 1..12: note = 21-4E3-C8-A HCDR3
SRSTLYSYDDGS

SEQ ID NO: 63 - protein, 6 aa, synthetic construct
  REGION 1..6: note = 21-4E3-C8-B LCDR1
QEISGD

SEQ ID NO: 64 - skipped

SEQ ID NO: 65 - protein, 9 aa, synthetic construct
  REGION 1..9: note = 21-4E3-C8-B LCDR3
LQYVSYPFT

SEQ ID NO: 66 - protein, 8 aa, synthetic construct
  REGION 1..8: note = 21-4E3-C8-B HCDR1
DYTFTDFY

SEQ ID NO: 67 - protein, 8 aa, synthetic construct
  REGION 1..8: note = 21-4E3-C8-B HCDR2
IYPLDDHT

SEQ ID NO: 68 - protein, 10 aa, synthetic construct
  REGION 1..10: note = 21-4E3-C8-B HCDR3
ARIYGYAMDY

SEQ ID NO: 69 - protein, 6 aa, synthetic construct
  REGION 1..6: note = 21-2H9-G2 LCDR1
QEISGD

SEQ ID NO: 70 - skipped

SEQ ID NO: 71 - protein, 9 aa, synthetic construct
  REGION 1..9: note = 21-2H9-G2 LCDR3
LQYVSYPFT

SEQ ID NO: 72 - protein, 9 aa, synthetic construct
  REGION 1..9: note = 21-2H9-G2 HCDR1
GYTFTSYWI

SEQ ID NO: 73 - protein, 8 aa, synthetic construct
  REGION 1..8: note = 21-2H9-G2 HCDR2
IYPGSGST

SEQ ID NO: 74 - protein, 12 aa, synthetic construct
  REGION 1..12: note = 21-2H9-G2 HCDR3
SRSTLYSYDDGS

SEQ ID NO: 75 - protein, 6 aa, synthetic construct
  REGION 1..6: note = 21-4G4-B11 LCDR1
SGCEYC

SEQ ID NO: 76 - skipped

SEQ ID NO: 77 - protein, 9 aa, synthetic construct
  REGION 1..9: note = 21-4G4-B11 LCDR3
QQHYITPWT

SEQ ID NO: 78 - protein, 8 aa, synthetic construct
  REGION 1..8: note = 21-4G4-B11 HCDR1
DYTFTDFY

SEQ ID NO: 79 - protein, 8 aa, synthetic construct
  REGION 1..8: note = 21-4G4-B11 HCDR2
IYPLDDHT

SEQ ID NO: 80 - protein, 10 aa, synthetic construct
  REGION 1..10: note = 21-4G4-B11 HCDR3
ARIYGYAMDY

SEQ ID NO: 81 - protein, 11 aa, synthetic construct
  REGION 1..11: note = 21-4B10-E1 LCDR1
IESPAIIWRHL

SEQ ID NO: 82 - skipped

SEQ ID NO: 83 - protein, 9 aa, synthetic construct
  REGION 1..9: note = 21-4B10-E1 LCDR3
YATSTISFH

SEQ ID NO: 84 - protein, 8 aa, synthetic construct
  REGION 1..8: note = 21-4B10-E1 HCDR1
GYSFTGYN

SEQ ID NO: 85 - protein, 8 aa, synthetic construct
  REGION 1..8: note = 21-4B10-E1 HCDR2
INPYFGSP

SEQ ID NO: 86 - protein, 13 aa, synthetic construct
  REGION 1..13: note = 21-4B10-E1 HCDR3
ASRQLGLGDTMDY

SEQ ID NO: 87 - protein, 6 aa, synthetic construct
  REGION 1..6: note = 22-2E9-G12 LCDR1
QNVNTN

SEQ ID NO: 88 - skipped

SEQ ID NO: 89 - protein, 9 aa, synthetic construct
  REGION 1..9: note = 22-2E9-G12 LCDR3
QQYIGYPYT

SEQ ID NO: 90 - protein, 8 aa, synthetic construct
  REGION 1..8: note = 22-2E9-G12-A HCDR1
GYTFINYW

SEQ ID NO: 91 - protein, 7 aa, synthetic construct
  REGION 1..7: note = 22-2E9-G12-A HCDR2
INPNCGV

SEQ ID NO: 92 - protein, 17 aa, synthetic construct
  REGION 1..17: note = 22-2E9-G12-A HCDR3
PHLLLRWLLHVPFAMVY

SEQ ID NO: 93 - protein, 8 aa, synthetic construct
  REGION 1..8: note = 22-2E9-G12-B HCDR1
GFNFNTYA

SEQ ID NO: 94 - protein, 10 aa, synthetic construct
  REGION 1..10: note = 22-2E9-G12-B HCDR2
IRTKSNSYAT

SEQ ID NO: 95 - protein, 9 aa, synthetic construct
  REGION 1..9: note = 22-2E9-G12-B HCDR3
VVTYWGFIY

SEQ ID NO: 96 - protein, 11 aa, synthetic construct
  REGION 1..11: note = 22-3E6-B11 LCDR1
QSLLYSDRKTY

SEQ ID NO: 97 - skipped

SEQ ID NO: 98 - protein, 9 aa, synthetic construct
  REGION 1..9: note = 22-3E6-B11 LCDR3
WQGTHFPQT

SEQ ID NO: 99 - protein, 8 aa, synthetic construct
  REGION 1..8: note = 22-3E6-B11 HCDR1
GYSFTAYY

SEQ ID NO: 100 - protein, 8 aa, synthetic construct
  REGION 1..8: note = 22-3E6-B11 HCDR2
INPSTDDT

SEQ ID NO: 101 - protein, 8 aa, synthetic construct
  REGION 1..8: note = 22-3E6-B11 HCDR3
ARYGEGAY

SEQ ID NO: 102 - protein, 11 aa, synthetic construct
  REGION 1..11: note = 22-4B11-B9 LCDR1
QSLLYSDGKTY

SEQ ID NO: 103 - skipped

SEQ ID NO: 104 - protein, 9 aa, synthetic construct
  REGION 1..9: note = 22-4B11-B9 LCDR3
WQGTHFPQT

SEQ ID NO: 105 - protein, 8 aa, synthetic construct
  REGION 1..8: note = 22-4B11-B9 HCDR1
GYSFTGFP

SEQ ID NO: 106 - protein, 7 aa, synthetic construct
  REGION 1..7: note = 22-4B11-B9 HCDR2
ISIYWWY

SEQ ID NO: 107 - protein, 8 aa, synthetic construct
  REGION 1..8: note = 22-4B11-B9 HCDR3
CKIRRGGL

SEQ ID NO: 108 - protein, 6 aa, synthetic construct
  REGION 1..6: note = 22-5B1-B2 LCDR1
ENVGTY

SEQ ID NO: 109 - skipped

SEQ ID NO: 110 - protein, 9 aa, synthetic construct
  REGION 1..9: note = 22-5B1-B2 LCDR3
GQSYSYPLT

SEQ ID NO: 111 - protein, 8 aa, synthetic construct
  REGION 1..8: note = 22-5B1-B2 HCDR1
GYSFTGYY

SEQ ID NO: 112 - protein, 8 aa, synthetic construct
  REGION 1..8: note = 22-5B1-B2 HCDR2
VNPISGGT

SEQ ID NO: 113 - protein, 8 aa, synthetic construct
  REGION 1..8: note = 22-5B1-B2 HCDR3
ARYGATDY

SEQ ID NO: 114 - protein, 8 aa, synthetic construct
  REGION 1..8: note = 22-5F2-E10 LCDR1
GYSFTGYY

SEQ ID NO: 115 - protein, 8 aa, synthetic construct
  REGION 1..8: note = 22-5F2-E10 LCDR2
INPTTGGT

SEQ ID NO: 116 - protein, 8 aa, synthetic construct
  REGION 1..8: note = 22-5F2-E10 LCDR3
ARYGEGAY

SEQ ID NO: 117 - protein, 11 aa, synthetic construct
  REGION 1..11: note = 22-5F2-E10 HCDR1
QSLFIITWKDI

SEQ ID NO: 118 - skipped

SEQ ID NO: 119 - protein, 8 aa, synthetic construct
  REGION 1..8: note = 22-5F2-E10 HCDR3
GKVHIFLR